European Patent Application EP 4 814 040 A1, published September 30, 2026. Title: Biologisch abbaubare Polyesterpolyurethane durch Enzymeinbau. Applicant: Covestro Deutschland AG. Application EP. The sequence listing filed with the application follows.

SEQUENCE LISTING (10 sequences)

SEQ ID NO: 1 - protein, 284 aa, Synthetic construct
MMANPYERGPNPTXSXLEAAXGPFSVATETVSRLSASGFGGGTIYYPXETSXTFGAVAISPGYTAXXXSIAWLGERIASHGFVVITIDTXTRLDXPDSRAXQLXAALNXLRXRSXSXVRXRJDXNRLAVMGHSMGGGGTLRJAXQXPSLKAAIPLTPWHXDKXWSSVXVPTLIXGAELDTIAPVSTHAKPFYNSLPSSXPKAYXELCGAXHFAPNIPNXXIXKYSIXWLKRFVDNDTRYXQFLCPXPDDXXXCEYRSTCPFCQGELEGKPIPNPLLGLDSTRTG

SEQ ID NO: 2 - protein, 263 aa, Thermobifida cellulosilytica
MANPYERGPNPTDALLEASSGPFSVSEENVSRLSASGFGGGTIYYPRENNTYGAVAISPGYTGTEASIAWLGERIASHGFVVITIDTITTLDQPDSRAEQLNAALNHMINRASSTVRSRIDSSRLAVMGHSMGGGGTLRLASQRPDLKAAIPLTPWHLNKNWSSVTVPTLIIGADLDTIAPVATHAKPFYNSLPSSISKAYLELDGATHFAPNIPNKIIGKYSVAWLKRFVDNDTRYTQFLCPGPRDGLFGEVEEYRSTCPFA

SEQ ID NO: 3 - protein, 263 aa, Thermobifida cellulosilytica
MANPYERGPNPTDALLEASSGPFSVSEENVSRLSASGFGGGTIYYPRENNTYGAVAISPGYTATEASIAWLGERIASHGFVVITIDTITTLDGPDSRAEQLNAALNHMINRASSTVRSRIDSSRLAVMGHSMGGGGTLRLASQRPDLKAAIPLTPWHLNKNWSSVTVPTLIIGADLDTIAPVATHAKPFYNSLPSSISKAYLELCGATHFAPNIPNKIIGKYSVAWLKRFVDNDTRYTQFLCPGPRDGLFGEVCEYRSTCPFA

SEQ ID NO: 4 - protein, 261 aa, Saccharomonospora viridis
MQDNPYERGPDPTEDSIEAIRGPFSVATERVSSFASGFGGGTIYYPRETDEGTFGAVAVAPGFTASQGSMSWYGERVASHGFIVFTIDTNTRLDAPGQRGRQLLAALDYLVERSDRKVRERLDPNRLAVMGHSMGGGGSLEATVMRPSLKASIPLTPWHLDKTWGQVQVPTFIIGAELDTIAPVSTHAKPFYESLPSSLPKAYMELCGATHFAPNIPNTTIAKYVISWLKRFVDEDTRYSQFLCPNPTDRAICEYRSTCPY

SEQ ID NO: 5 - protein, 196 aa, Thermomyces insolens
MGQLGAIENGLESGSANACPDAILIFARGSTEPGNMGITVGPALANGLESHIRNIWIQGVGGPYDAALATNFLPRGTSQANIDEGKRLFALANQKCPNTPVVAGGYSQGAALIAAAVSELSGAVKEQVKGVALFGYTQNLQNRGGIPNYPRERTKVFCNVGDAVCTGTLIITPAHLSYTIEARGEAARFLRDRIRA

SEQ ID NO: 6 - protein, 259 aa, synthetic construct
MANPYERGPDPTESSIEAVRGPFAVAQTTVSRLQADGFGGGTIYYPTDTSQGTFGAVAISPGFTAGQESIAWLGPRIASQGFVVITIDTITRLDQPDSRGRQLQAALDHLRTNSVVRNRIDPNRMAVMGHSMGGGGALSAAANNTSLEAAIPLQGWHTRKNWSSVRTPTLVVGAQLDTIAPVSSHSEAFYNSLPSDLDKAYMELRGASHLVSNTPDTTTAKYSIAWLKRFVDDDLRYEQFLCPAPDDFAISEYRSTCPF

SEQ ID NO: 7 - protein, 297 aa, Thermobifida fusca
MGSGSGDDDDKLAANPYERGPNPTDALLEARSGPFSVSEENVSRLSASGFGGGTIYYPRENNTYGAVAISPGYTGTEASIAWLGERIASHGFVVITIDTITTLDQPDSRAEQLNAALNHMINRASSTVRSRIDSSRLAVMGHSMGGGGSLRLASQRPDLKAAIPLTPWHLNKNWSSVTVPTLIIGADLDTIAPVATHAKPFYNSLPSSISKAYLELDGATHFAPNIPNKIIGKYSVAWLKRFVDNDTRYTQFLCPGPRDGLFGEVEEYRSTCPFYKGELEGKPIPNPLLGLDSTRTG

SEQ ID NO: 8 - protein, 259 aa, synthetic construct
MSNPYQRGPNPTRSALTADGPFSVATYTVSRLSVSGFGGGVIYYPTGTSLTFGGIAMSPGYTADASSLAWLGRRLASHGFVVLVINTNSRFDYPDSRASQLSAALNYLRTSSPSAVRARLDANRLAVAGHSMGGGGTLRIAEQNPSLKAAVPLTPWHTDKTFNTSVPVLIVGAEADTVAPVSQHAIPFYQNLPSTTPKVYVELDNASHFAPNSNNAAISVYTISWMKLWVDNDTRYRQFLCNVNDPALSDFRTNNRHCQ

SEQ ID NO: 9 - protein, 259 aa, synthetic construct
MSNPYQRGPNPTRSALTADGPFSVATYTVSRLSVSGFGGGVIYYPTGTSLTFGGIAMSPGYTADASSLAWLGRRLASHGFVVLVINTNSRFDGPDSRASQLSAALNYLRTSSPSAVRARLDANRLAVAGHSMGGGGTLRIAEQNPSLKAAVPLTPWHTDKTFNTSVPVLIVGAEADTVAPVSQHAIPFYQNLPSTTPKVYVELCNASHWAPNSNNAAISVYTISWMKLWVDNDTRYRQFLCNVNDPALCDFRTNNRHCQ

SEQ ID NO: 10 - protein, 259 aa, synthetic construct
MSNPYQRGPNPTRSALTADGPFSVATYTVSRLSVSGFGGGVIYYPTGTSLTFGGIAMSPGYTADASSLAWLGRRLASHGFVVLVINTNSRFDGPDSRASQLSAALNYLRTSSPSAVRARLDANRLAVAGHSMGGGGTLRIAEQNPSLKAAVPLTPWHTDKTFNTSVPVLIVGAEADTVAPVSQHAIPFYQNLPSTTPKVYVELCNASHIAPNSNNAAISVYTISWMKLWVDNDTRYRQFLCNVNDPALCDFRTNNRHCQ